European Patent Application EP 4 446 342 A1, published October 16, 2024. Title: 包含LRRC15抗原结合结构域的多特异性T细胞接合剂. Applicant: 苏州泽璟生物制药股份有限公司. The sequence listing filed with the application follows.

SEQUENCE LISTING (88 sequences)

SEQ ID NO: 1 - protein, 127 aa, synthetic construct
  source 1..127: note = VH; L15-06H
EVQLLESGGGLVQPGGSLRLSCAASGFTFSSYYMSWVRQAPGKGLEWVADISVSGSYTNYADSVKGRFTISRDNSKNTLYLQMNSLRAEDTAVYYCARIGSYRSFFSTDDGDSLDYWGQGTLVTVSS

SEQ ID NO: 2 - protein, 127 aa, synthetic construct
  source 1..127: note = VH; L15-08H
QVQLVESGGGLVKPGGSLRLSCAASGFTFSDYYMSWIRQAPGKGLEWVSDISVSSSYTNYADSVKGRFTISRDNAKNSLYLQMNSLRAEDTAVYYCARLGGYRSFFSTDDGDSLDYWGQGTLVTVSS

SEQ ID NO: 3 - protein, 120 aa, synthetic construct
  source 1..120: note = VH; L15-03H
QVQLVQSGAEVKKPGSSVKVSCKASGGTFSSYTISWVRQAPGQGLEWMGGIIPMFGTANYAQKFQGRVTITADESTSTAYMELSSLRSEDTAVYYCARGVALLATDFDYWGQGTLVTVSS

SEQ ID NO: 4 - protein, 119 aa, synthetic construct
  source 1..119: note = VH; L15-07H
QVQLVQSGAEVKKPGSSVKVSCKASGGTFSTYAISWVRQAPGQGLEWMGGITPMFGTPNYAQKFQGRVTITADESTSTAYMELSSLRSEDTAVYYCARGDWYDYHFDYWGQGTLVTVSS

SEQ ID NO: 5 - protein, 107 aa, synthetic construct
  source 1..107: note = VL; L15-06L
DIQMTQSPSTLSASVGDRVTITCRASQSISSWLAWYQQKPGKAPKLLIYDASSLESGVPSRFSGSGSGTEFTLTISSLQPDDFATYYCQQYNSYSLTFGGGTKVEIK

SEQ ID NO: 6 - protein, 107 aa, synthetic construct
  source 1..107: note = VL; L15-08L
DIQLTQSPSTLSASVGDRVTITCRASQSISSWLAWYQQKPGKAPKLLIYDAFSLESGVPSRFSGSGSGTEFTLTISSLQPDDFATYYCQQYNSYSITFGGGTKVEIK

SEQ ID NO: 7 - protein, 110 aa, synthetic construct
  source 1..110: note = VL; L15-03L
QSALTQPASVSGSPGQSITISCTGTSSDVGGYNYVSWYQQHPGKAPKLMIYEVSNRPSGVSNRFSGSKSGNTASLTISGLQAEDEADYYCQSWTHDNSVVFGGGTKLTVL

SEQ ID NO: 8 - protein, 111 aa, synthetic construct
  source 1..111: note = VL; L15-07L
QSALTQPASVSGSPGQSITISCTGTSSDVGGYNYVSWYQQHPGKAPKLMIYEVSNRPSGVSNRFSGSKSGNTASLTISGLQAEDEADYYCQSYANRDNFVVFGGGTKLTVL

SEQ ID NO: 9 - protein, 125 aa, synthetic construct
  source 1..125: note = VH; CD3vB
EVQLVESGGGLVQPGGSLRLSCAASGFTFSTYAMNWVRQAPGKGLEWVGRIRSKANNYATYYADSVKGRFTISRDDSKNTLYLQMNSLRAEDTAVYYCVRHGNFGDSYVSWFAYWGQGTLVTVSS

SEQ ID NO: 10 - protein, 125 aa, synthetic construct
  source 1..125: note = VH; CD3vG
EVQLVESGGGLVQPGGSLRLSCAASGFTFSTYAMNWVRQAPGKGLEWVGRIRSKSNNYATYYADSVKGRFTISRDDSKNTLYLQMNSLRAEDTAVYYCVRHGNFGDSYVSWFAYWGQGTLVTVSS

SEQ ID NO: 11 - protein, 125 aa, synthetic construct
  source 1..125: note = VH; CD3vI
EVQLVESGGGLVQPGGSLRLSCAASGFTFSTYAMNWVRQAPGKGLEWVGRIRSKYNNYATYYADSVKGRFTISRDDSKNTLYLQMNSLRAEDTAVYYCVRHGNFGDSYVSWFEYWGQGTLVTVSS

SEQ ID NO: 12 - protein, 125 aa, synthetic construct
  source 1..125: note = VH; CD3vJ
EVQLVESGGGLVQPGGSLRLSCAASGFTFSTYAMNWVRQAPGKGLEWVGRIRSKYNNYATYYADSVKGRFTISRDDSKNTLYLQMNSLRAEDTAVYYCVRHGNFGDSYVSWFDYWGQGTLVTVSS

SEQ ID NO: 13 - protein, 109 aa, synthetic construct
  source 1..109: note = VL; CD3
QAVVTQEPSLTVSPGGTVTLTCGSSTGAVTTSNYANWVQQKPGKSPRGLIGGTNKRAPGVPARFSGSLLGGKAALTISGAQPEDEADYYCALWYSNHWVFGGGTKLTVL

SEQ ID NO: 14 - protein, 120 aa, synthetic construct
  source 1..120: note = VH;CD28 (C50S)
QVQLVQSGAEVKKPGASVKVSCKASGYTFTSYYIHWVRQAPGQGLEWIGSIYPGNVNTNYNEKFKDRATLTVDTSISTAYMELSRLRSDDTAVYFCTRSHYGLDWNFDVWGQGTTVTVSS

SEQ ID NO: 15 - protein, 107 aa, synthetic construct
  source 1..107: note = VL; CD28
DIQMTQSPSSLSASVGDRVTITCHASQNIYVWLNWYQQKPGKAPKLLIYKASNLHTGVPSRFSGSGSGTDFTLTISSLQPEDFATYYCQQGQTYPYTFGGGTKVEIK

SEQ ID NO: 16 - protein, 126 aa, synthetic construct
  source 1..126: note = VH; CD40
QVQLVQSGAEVKKPGASVKVSCKASGYTFTGYYMHWVRQAPGQGLEWMGWINPDSGGTNYAQKFQGRVTMTRDTSISTAYMELNRLRSDDTAVYYCARDQPLGYCTNGVCSYFDYWGQGTLVTVSS

SEQ ID NO: 17 - protein, 107 aa, synthetic construct
  source 1..107: note = VL; CD40
DIQMTQSPSSVSASVGDRVTITCRASQGIYSWLAWYQQKPGKAPNLLIYTASTLQSGVPSRFSGSGSGTDFTLTISSLQPEDFATYYCQQANIFPLTFGGGTKVEIK

SEQ ID NO: 18 - protein, 121 aa, synthetic construct [sequence omitted]

SEQ ID NO: 19 - protein, 109 aa, synthetic construct [sequence omitted]

SEQ ID NO: 20 - protein, 116 aa, synthetic construct
  source 1..116: note = VH; CD137o
EVQLVQSGAEVKKPGESLRISCKGSGYSFSTYWISWVRQMPGKGLEWMGKIYPGDSYTNYSPSFQGQVTISADKSISTAYLQWSSLKASDTAMYYCARGYGIFDYWGQGTLVTVSS

SEQ ID NO: 21 - protein, 108 aa, synthetic construct
  source 1..108: note = VL; CD137o
SYELTQPPSVSVSPGQTASITCSGDNIGDQYAHWYQQKPGQSPVLVIYQDKNRPSGIPERFSGSNSGNTATLTISGTQAMDEADYYCATYTGFGSLAVFGGGTKLTVL

SEQ ID NO: 22 - protein, 215 aa, synthetic construct
  source 1..215: note = CD40LECD (47-261)
HRRLDKIEDERNLHEDFVFMKTIQRCNTGERSLSLLNCEEIKSQFEGFVKDIMLNKEETKKENSFEMQKGDQNPQIAAHVISEASSKTTSVLQWAEKGYYTMSNNLVTLENGKQLTVKRQGLYYIYAQVTFCSNREASSQAPFIASLCLKSPGRFERILLRAANTHSSAKPCGQQSIHLGGVFELQPGASVFVNVTDPSQVSHGTGFTSFGLLKL

SEQ ID NO: 23 - protein, 143 aa, synthetic construct
  source 1..143: note = CD40LRBD(119-261)
NPQIAAHVISEASSKTTSVLQWAEKGYYTMSNNLVTLENGKQLTVKRQGLYYIYAQVTFCSNREASSQAPFIASLCLKSPGRFERILLRAANTHSSAKPCGQQSIHLGGVFELQPGASVFVNVTDPSQVSHGTGFTSFGLLKL

SEQ ID NO: 24 - protein, 205 aa, synthetic construct
  source 1..205: note = CD137LECD (50-254)
ACPWAVSGARASPGSAASPRLREGPELSPDDPAGLLDLRQGMFAQLVAQNVLLIDGPLSWYSDPGLAGVSLTGGLSYKEDTKELVVAKAGVYYVFFQLELRRVVAGEGSGSVSLALHLQPLRSAAGAAALALTVDLPPASSEARNSAFGFQGRLLHLSAGQRLGVHLHTEARARHAWQLTQGATVLGLFRVTPEIPAGLPSPRSE

SEQ ID NO: 25 - protein, 184 aa, synthetic construct
  source 1..184: note = CD137LRBD (71-254)
REGPELSPDDPAGLLDLRQGMFAQLVAQNVLLIDGPLSWYSDPGLAGVSLTGGLSYKEDTKELVVAKAGVYYVFFQLELRRVVAGEGSGSVSLALHLQPLRSAAGAAALALTVDLPPASSEARNSAFGFQGRLLHLSAGQRLGVHLHTEARARHAWQLTQGATVLGLFRVTPEIPAGLPSPRSE

SEQ ID NO: 26 - protein, 98 aa, Homo sapiens
ASTKGPSVFPLAPSSKSTSGGTAALGCLVKDYFPEPVTVSWNSGALTSGVHTFPAVLQSSGLYSLSSVVTVPSSSLGTQTYICNVNHKPSNTKVDKRV

SEQ ID NO: 27 - protein, 232 aa, Homo sapiens
EPKSCDKTHTCPPCPAPELLGGPSVFLFPPKPKDTLMISRTPEVTCVVVDVSHEDPEVKFNWYVDGVEVHNAKTKPREEQYNSTYRVVSVLTVLHQDWLNGKEYKCKVSNKALPAPIEKTISKAKGQPREPQVYTLPPSRDELTKNQVSLTCLVKGFYPSDIAVEWESNGQPENNYKTTPPVLDSDGSFFLYSKLTVDKSRWQQGNVFSCSVMHEALHNHYTQKSLSLSPGK

SEQ ID NO: 28 - protein, 98 aa, Homo sapiens
ASTKGPSVFPLAPCSRSTSESTAALGCLVKDYFPEPVTVSWNSGALTSGVHTFPAVLQSSGLYSLSSVVTVPSSSLGTKTYTCNVDHKPSNTKVDKRV

SEQ ID NO: 29 - protein, 229 aa, Homo sapiens
ESKYGPPCPPCPAPEFLGGPSVFLFPPKPKDTLMISRTPEVTCVVVDVSQEDPEVQFNWYVDGVEVHNAKTKPREEQFNSTYRVVSVLTVLHQDWLNGKEYKCKVSNKGLPSSIEKTISKAKGQPREPQVYTLPPSQKKMTKNQVSLTCLVKGFYPSDIAVEWESNGQPENNYKTTPPVLKSDGSFFLYSRLTVDKSRWQEGNVFSCSVMHEALHNHYTQKSLSLSLGK

SEQ ID NO: 30 - protein, 107 aa, Homo sapiens [sequence omitted]

SEQ ID NO: 31 - protein, 106 aa, Homo sapiens
GQPKAAPSVTLFPPSSEELQANKATLVCLISDFYPGAVTVAWKADSSPVKAGVETTTPSKQSNNKYAASSYLSLTPEQWKSHRSYSCQVTHEGSTVEKTVAPTECS

SEQ ID NO: 32 - protein, 10 aa, synthetic construct
  source 1..10: note = HCDR1; L15-06H/ L15-06CH
GFTFSSYYMS

SEQ ID NO: 33 - protein, 17 aa, synthetic construct
  source 1..17: note = HCDR2; L15-06H/ L15-06CH
DISVSGSYTNYADSVKG

SEQ ID NO: 34 - protein, 18 aa, synthetic construct
  source 1..18: note = HCDR3; L15-06H/ L15-06CH
IGSYRSFFSTDDGDSLDY

SEQ ID NO: 35 - protein, 10 aa, synthetic construct
  source 1..10: note = HCDR1; L15-08H
GFTFSDYYMS

SEQ ID NO: 36 - protein, 17 aa, synthetic construct
  source 1..17: note = HCDR2; L15-08H
DISVSSSYTNYADSVKG

SEQ ID NO: 37 - protein, 18 aa, synthetic construct
  source 1..18: note = HCDR3; L15-08H
LGGYRSFFSTDDGDSLDY

SEQ ID NO: 38 - protein, 10 aa, synthetic construct
  source 1..10: note = HCDR1; L15-03H
GGTFSSYTIS

SEQ ID NO: 39 - protein, 17 aa, synthetic construct
  source 1..17: note = HCDR2; L15-03H
GIIPMFGTANYAQKFQG

SEQ ID NO: 40 - protein, 11 aa, synthetic construct
  source 1..11: note = HCDR3; L15-03H
GVALLATDFDY

SEQ ID NO: 41 - protein, 10 aa, synthetic construct
  source 1..10: note = HCDR1; L15-07H
GGTFSTYAIS

SEQ ID NO: 42 - protein, 17 aa, synthetic construct
  source 1..17: note = HCDR2; L15-07H
GITPMFGTPNYAQKFQG

SEQ ID NO: 43 - protein, 10 aa, synthetic construct
  source 1..10: note = HCDR3; L15-07H
GDWYDYHFDY

SEQ ID NO: 44 - protein, 11 aa, synthetic construct
  source 1..11: note = LCDR1; L15-06L/ L15-06CL/L15-08L
RASQSISSWLA

SEQ ID NO: 45 - protein, 7 aa, synthetic construct
  source 1..7: note = LCDR2; L15-06L/ L15-06CL
DASSLES

SEQ ID NO: 46 - protein, 9 aa, synthetic construct
  source 1..9: note = LCDR3; L15-06L/ L15-06CL
QQYNSYSLT

SEQ ID NO: 47 - protein, 7 aa, synthetic construct
  source 1..7: note = LCDR2; L15-08L
DAFSLES

SEQ ID NO: 48 - protein, 9 aa, synthetic construct
  source 1..9: note = LCDR3; L15-08L
QQYNSYSIT

SEQ ID NO: 49 - protein, 14 aa, synthetic construct
  source 1..14: note = LCDR1; L15-03L/L15-07L
TGTSSDVGGYNYVS

SEQ ID NO: 50 - protein, 7 aa, synthetic construct
  source 1..7: note = LCDR2; L15-03L/L15-07L
EVSNRPS

SEQ ID NO: 51 - protein, 10 aa, synthetic construct
  source 1..10: note = LCDR3; L15-03L
QSWTHDNSVV

SEQ ID NO: 52 - protein, 11 aa, synthetic construct
  source 1..11: note = LCDR3; L15-07L
QSYANRDNFVV

SEQ ID NO: 53 - protein, 127 aa, synthetic construct
  source 1..127: note = VH; L15-06CH
EVQLLESGGGLVQPGGSLRLSCAASGFTFSSYYMSWVRQAPGKCLEWVADISVSGSYTNYADSVKGRFTISRDNSKNTLYLQMNSLRAEDTAVYYCARIGSYRSFFSTDDGDSLDYWGQGTLVTVSS

SEQ ID NO: 54 - protein, 107 aa, synthetic construct
  source 1..107: note = VL; L15-06CL
DIQMTQSPSTLSASVGDRVTITCRASQSISSWLAWYQQKPGKAPKLLIYDASSLESGVPSRFSGSGSGTEFTLTISSLQPDDFATYYCQQYNSYSLTFGCGTKVEIK

SEQ ID NO: 55 - protein, 114 aa, synthetic construct [sequence omitted]

SEQ ID NO: 56 - protein, 112 aa, synthetic construct [sequence omitted]

SEQ ID NO: 57 - protein, 232 aa, synthetic construct
  source 1..232: note = Fc(C220S/L234F/L235E/P331S/S354C/D356K/E357K/D399K)
EPKSSDKTHTCPPCPAPEFEGGPSVFLFPPKPKDTLMISRTPEVTCVVVDVSHEDPEVKFNWYVDGVEVHNAKTKPREEQYNSTYRVVSVLTVLHQDWLNGKEYKCKVSNKALPASIEKTISKAKGQPREPQVYTLPPCRKKLTKNQVSLTCLVKGFYPSDIAVEWESNGQPENNYKTTPPVLKSDGSFFLYSKLTVDKSRWQQGNVFSCSVMHEALHNHYTQKSLSLSPGK

SEQ ID NO: 58 - protein, 232 aa, synthetic construct
  source 1..232: note = Fc(L234F/L235E/P331S/Y349C/K370E/K409D/K439E)
EPKSCDKTHTCPPCPAPEFEGGPSVFLFPPKPKDTLMISRTPEVTCVVVDVSHEDPEVKFNWYVDGVEVHNAKTKPREEQYNSTYRVVSVLTVLHQDWLNGKEYKCKVSNKALPASIEKTISKAKGQPREPQVCTLPPSRDELTKNQVSLTCLVEGFYPSDIAVEWESNGQPENNYKTTPPVLDSDGSFFLYSDLTVDKSRWQQGNVFSCSVMHEALHNHYTQESLSLSPGK

SEQ ID NO: 59 - protein, 232 aa, synthetic construct
  source 1..232: note = Fc(L234F/L235E/S267E/P331S)
EPKSCDKTHTCPPCPAPEFEGGPSVFLFPPKPKDTLMISRTPEVTCVVVDVEHEDPEVKFNWYVDGVEVHNAKTKPREEQYNSTYRVVSVLTVLHQDWLNGKEYKCKVSNKALPASIEKTISKAKGQPREPQVYTLPPSRDELTKNQVSLTCLVKGFYPSDIAVEWESNGQPENNYKTTPPVLDSDGSFFLYSKLTVDKSRWQQGNVFSCSVMHEALHNHYTQKSLSLSPGK

SEQ ID NO: 60 - protein, 232 aa, synthetic construct
  source 1..232: note = Fc(L234F/L235E/P331S)
EPKSCDKTHTCPPCPAPEFEGGPSVFLFPPKPKDTLMISRTPEVTCVVVDVSHEDPEVKFNWYVDGVEVHNAKTKPREEQYNSTYRVVSVLTVLHQDWLNGKEYKCKVSNKALPASIEKTISKAKGQPREPQVYTLPPSRDELTKNQVSLTCLVKGFYPSDIAVEWESNGQPENNYKTTPPVLDSDGSFFLYSKLTVDKSRWQQGNVFSCSVMHEALHNHYTQKSLSLSPGK

SEQ ID NO: 61 - protein, 486 aa, synthetic construct
  source 1..486: note = chain 1
EVQLVESGGGLVQPGGSLRLSCAASGFTFSTYAMNWVRQAPGKGLEWVGRIRSKYNNYATYYADSVKGRFTISRDDSKNTLYLQMNSLRAEDTAVYYCVRHGNFGDSYVSWFEYWGQGTLVTVSSGGGGSGGGGSGGGGSGGGGSQAVVTQEPSLTVSPGGTVTLTCGSSTGAVTTSNYANWVQQKPGKSPRGLIGGTNKRAPGVPARFSGSLLGGKAALTISGAQPEDEADYYCALWYSNHWVFGGGTKLTVLEPKSSDKTHTCPPCPAPEFEGGPSVFLFPPKPKDTLMISRTPEVTCVVVDVSHEDPEVKFNWYVDGVEVHNAKTKPREEQYNSTYRVVSVLTVLHQDWLNGKEYKCKVSNKALPASIEKTISKAKGQPREPQVYTLPPCRKKLTKNQVSLTCLVKGFYPSDIAVEWESNGQPENNYKTTPPVLKSDGSFFLYSKLTVDKSRWQQGNVFSCSVMHEALHNHYTQKSLSLSPGK

SEQ ID NO: 62 - protein, 746 aa, synthetic construct
  source 1..746: note = chain 1
EVQLLESGGGLVQPGGSLRLSCAASGFTFSSYYMSWVRQAPGKGLEWVADISVSGSYTNYADSVKGRFTISRDNSKNTLYLQMNSLRAEDTAVYYCARIGSYRSFFSTDDGDSLDYWGQGTLVTVSSGGGGSGGGGSGGGGSGGGGSDIQMTQSPSTLSASVGDRVTITCRASQSISSWLAWYQQKPGKAPKLLIYDASSLESGVPSRFSGSGSGTEFTLTISSLQPDDFATYYCQQYNSYSLTFGGGTKVEIKSGGGGSEVQLVESGGGLVQPGGSLRLSCAASGFTFSTYAMNWVRQAPGKGLEWVGRIRSKYNNYATYYADSVKGRFTISRDDSKNTLYLQMNSLRAEDTAVYYCVRHGNFGDSYVSWFEYWGQGTLVTVSSGKPGSGKPGSGKPGSGKPGSQAVVTQEPSLTVSPGGTVTLTCGSSTGAVTTSNYANWVQQKPGKSPRGLIGGTNKRAPGVPARFSGSLLGGKAALTISGAQPEDEADYYCALWYSNHWVFGGGTKLTVLEPKSSDKTHTCPPCPAPEFEGGPSVFLFPPKPKDTLMISRTPEVTCVVVDVSHEDPEVKFNWYVDGVEVHNAKTKPREEQYNSTYRVVSVLTVLHQDWLNGKEYKCKVSNKALPASIEKTISKAKGQPREPQVYTLPPCRKKLTKNQVSLTCLVKGFYPSDIAVEWESNGQPENNYKTTPPVLKSDGSFFLYSKLTVDKSRWQQGNVFSCSVMHEALHNHYTQKSLSLSPGK

SEQ ID NO: 63 - protein, 742 aa, synthetic construct
  source 1..742: note = chain 1
QVQLVQSGAEVKKPGSSVKVSCKASGGTFSTYAISWVRQAPGQGLEWMGGITPMFGTPNYAQKFQGRVTITADESTSTAYMELSSLRSEDTAVYYCARGDWYDYHFDYWGQGTLVTVSSGGGGSGGGGSGGGGSGGGGSQSALTQPASVSGSPGQSITISCTGTSSDVGGYNYVSWYQQHPGKAPKLMIYEVSNRPSGVSNRFSGSKSGNTASLTISGLQAEDEADYYCQSYANRDNFVVFGGGTKLTVLSGGGGSEVQLVESGGGLVQPGGSLRLSCAASGFTFSTYAMNWVRQAPGKGLEWVGRIRSKYNNYATYYADSVKGRFTISRDDSKNTLYLQMNSLRAEDTAVYYCVRHGNFGDSYVSWFEYWGQGTLVTVSSGKPGSGKPGSGKPGSGKPGSQAVVTQEPSLTVSPGGTVTLTCGSSTGAVTTSNYANWVQQKPGKSPRGLIGGTNKRAPGVPARFSGSLLGGKAALTISGAQPEDEADYYCALWYSNHWVFGGGTKLTVLEPKSSDKTHTCPPCPAPEFEGGPSVFLFPPKPKDTLMISRTPEVTCVVVDVSHEDPEVKFNWYVDGVEVHNAKTKPREEQYNSTYRVVSVLTVLHQDWLNGKEYKCKVSNKALPASIEKTISKAKGQPREPQVYTLPPCRKKLTKNQVSLTCLVKGFYPSDIAVEWESNGQPENNYKTTPPVLKSDGSFFLYSKLTVDKSRWQQGNVFSCSVMHEALHNHYTQKSLSLSPGK

SEQ ID NO: 64 - protein, 746 aa, synthetic construct
  source 1..746: note = chain 1
EVQLLESGGGLVQPGGSLRLSCAASGFTFSSYYMSWVRQAPGKCLEWVADISVSGSYTNYADSVKGRFTISRDNSKNTLYLQMNSLRAEDTAVYYCARIGSYRSFFSTDDGDSLDYWGQGTLVTVSSGGGGSGGGGSGGGGSGGGGSDIQMTQSPSTLSASVGDRVTITCRASQSISSWLAWYQQKPGKAPKLLIYDASSLESGVPSRFSGSGSGTEFTLTISSLQPDDFATYYCQQYNSYSLTFGCGTKVEIKSGGGGSEVQLVESGGGLVQPGGSLRLSCAASGFTFSTYAMNWVRQAPGKGLEWVGRIRSKYNNYATYYADSVKGRFTISRDDSKNTLYLQMNSLRAEDTAVYYCVRHGNFGDSYVSWFEYWGQGTLVTVSSGKPGSGKPGSGKPGSGKPGSQAVVTQEPSLTVSPGGTVTLTCGSSTGAVTTSNYANWVQQKPGKSPRGLIGGTNKRAPGVPARFSGSLLGGKAALTISGAQPEDEADYYCALWYSNHWVFGGGTKLTVLEPKSSDKTHTCPPCPAPEFEGGPSVFLFPPKPKDTLMISRTPEVTCVVVDVSHEDPEVKFNWYVDGVEVHNAKTKPREEQYNSTYRVVSVLTVLHQDWLNGKEYKCKVSNKALPASIEKTISKAKGQPREPQVYTLPPCRKKLTKNQVSLTCLVKGFYPSDIAVEWESNGQPENNYKTTPPVLKSDGSFFLYSKLTVDKSRWQQGNVFSCSVMHEALHNHYTQKSLSLSPGK

SEQ ID NO: 65 - protein, 746 aa, synthetic construct
  source 1..746: note = chain 1
QVQLVESGGGLVKPGGSLRLSCAASGFTFSDYYMSWIRQAPGKGLEWVSDISVSSSYTNYADSVKGRFTISRDNAKNSLYLQMNSLRAEDTAVYYCARLGGYRSFFSTDDGDSLDYWGQGTLVTVSSGGGGSGGGGSGGGGSGGGGSDIQLTQSPSTLSASVGDRVTITCRASQSISSWLAWYQQKPGKAPKLLIYDAFSLESGVPSRFSGSGSGTEFTLTISSLQPDDFATYYCQQYNSYSITFGGGTKVEIKSGGGGSEVQLVESGGGLVQPGGSLRLSCAASGFTFSTYAMNWVRQAPGKGLEWVGRIRSKYNNYATYYADSVKGRFTISRDDSKNTLYLQMNSLRAEDTAVYYCVRHGNFGDSYVSWFEYWGQGTLVTVSSGKPGSGKPGSGKPGSGKPGSQAVVTQEPSLTVSPGGTVTLTCGSSTGAVTTSNYANWVQQKPGKSPRGLIGGTNKRAPGVPARFSGSLLGGKAALTISGAQPEDEADYYCALWYSNHWVFGGGTKLTVLEPKSSDKTHTCPPCPAPEFEGGPSVFLFPPKPKDTLMISRTPEVTCVVVDVSHEDPEVKFNWYVDGVEVHNAKTKPREEQYNSTYRVVSVLTVLHQDWLNGKEYKCKVSNKALPASIEKTISKAKGQPREPQVYTLPPCRKKLTKNQVSLTCLVKGFYPSDIAVEWESNGQPENNYKTTPPVLKSDGSFFLYSKLTVDKSRWQQGNVFSCSVMHEALHNHYTQKSLSLSPGK

SEQ ID NO: 66 - protein, 746 aa, synthetic construct
  source 1..746: note = chain 1
QVQLVESGGGLVKPGGSLRLSCAASGFTFSDYYMSWIRQAPGKCLEWVSDISVSSSYTNYADSVKGRFTISRDNAKNSLYLQMNSLRAEDTAVYYCARLGGYRSFFSTDDGDSLDYWGQGTLVTVSSGGGGSGGGGSGGGGSGGGGSDIQLTQSPSTLSASVGDRVTITCRASQSISSWLAWYQQKPGKAPKLLIYDAFSLESGVPSRFSGSGSGTEFTLTISSLQPDDFATYYCQQYNSYSITFGCGTKVEIKSGGGGSEVQLVESGGGLVQPGGSLRLSCAASGFTFSTYAMNWVRQAPGKGLEWVGRIRSKYNNYATYYADSVKGRFTISRDDSKNTLYLQMNSLRAEDTAVYYCVRHGNFGDSYVSWFEYWGQGTLVTVSSGKPGSGKPGSGKPGSGKPGSQAVVTQEPSLTVSPGGTVTLTCGSSTGAVTTSNYANWVQQKPGKSPRGLIGGTNKRAPGVPARFSGSLLGGKAALTISGAQPEDEADYYCALWYSNHWVFGGGTKLTVLEPKSSDKTHTCPPCPAPEFEGGPSVFLFPPKPKDTLMISRTPEVTCVVVDVSHEDPEVKFNWYVDGVEVHNAKTKPREEQYNSTYRVVSVLTVLHQDWLNGKEYKCKVSNKALPASIEKTISKAKGQPREPQVYTLPPCRKKLTKNQVSLTCLVKGFYPSDIAVEWESNGQPENNYKTTPPVLKSDGSFFLYSKLTVDKSRWQQGNVFSCSVMHEALHNHYTQKSLSLSPGK

SEQ ID NO: 67 - protein, 739 aa, synthetic construct
  source 1..739: note = chain 1
QVQLVQSGAEVKKPGASVKVSCKASGYTFTSYYIHWVRQAPGQGLEWIGSIYPGNVNTNYNEKFKDRATLTVDTSISTAYMELSRLRSDDTAVYFCTRSHYGLDWNFDVWGQGTTVTVSSGGGGSGGGGSGGGGSGGGGSDIQMTQSPSSLSASVGDRVTITCHASQNIYVWLNWYQQKPGKAPKLLIYKASNLHTGVPSRFSGSGSGTDFTLTISSLQPEDFATYYCQQGQTYPYTFGGGTKVEIKSGGGGSEVQLVESGGGLVQPGGSLRLSCAASGFTFSTYAMNWVRQAPGKGLEWVGRIRSKYNNYATYYADSVKGRFTISRDDSKNTLYLQMNSLRAEDTAVYYCVRHGNFGDSYVSWFEYWGQGTLVTVSSGKPGSGKPGSGKPGSGKPGSQAVVTQEPSLTVSPGGTVTLTCGSSTGAVTTSNYANWVQQKPGKSPRGLIGGTNKRAPGVPARFSGSLLGGKAALTISGAQPEDEADYYCALWYSNHWVFGGGTKLTVLEPKSSDKTHTCPPCPAPEFEGGPSVFLFPPKPKDTLMISRTPEVTCVVVDVSHEDPEVKFNWYVDGVEVHNAKTKPREEQYNSTYRVVSVLTVLHQDWLNGKEYKCKVSNKALPASIEKTISKAKGQPREPQVYTLPPCRKKLTKNQVSLTCLVKGFYPSDIAVEWESNGQPENNYKTTPPVLKSDGSFFLYSKLTVDKSRWQQGNVFSCSVMHEALHNHYTQKSLSLSPGK

SEQ ID NO: 68 - protein, 610 aa, synthetic construct
  source 1..610: note = chain 1
EVQLLESGGGLVQPGGSLRLSCAASGFTFSSYYMSWVRQAPGKGLEWVADISVSGSYTNYADSVKGRFTISRDNSKNTLYLQMNSLRAEDTAVYYCARIGSYRSFFSTDDGDSLDYWGQGTLVTVSSASTKGPSVFPLAPSSKSTSGGTAALGCLVKDYFPEPVTVSWNSGALTSGVHTFPAVLQSSGLYSLSSVVTVPSSSLGTQTYICNVNHKPSNTKVDKRVEPKSCDKTHTCPPCPAPEFEGGPSVFLFPPKPKDTLMISRTPEVTCVVVDVEHEDPEVKFNWYVDGVEVHNAKTKPREEQYNSTYRVVSVLTVLHQDWLNGKEYKCKVSNKALPASIEKTISKAKGQPREPQVYTLPPSRDELTKNQVSLTCLVKGFYPSDIAVEWESNGQPENNYKTTPPVLDSDGSFFLYSKLTVDKSRWQQGNVFSCSVMHEALHNHYTQKSLSLSPGKGGGGSGGGGSNPQIAAHVISEASSKTTSVLQWAEKGYYTMSNNLVTLENGKQLTVKRQGLYYIYAQVTFCSNREASSQAPFIASLCLKSPGRFERILLRAANTHSSAKPCGQQSIHLGGVFELQPGASVFVNVTDPSQVSHGTGFTSFGLLKL

SEQ ID NO: 69 - protein, 916 aa, synthetic construct
  source 1..916: note = chain 1
EVQLLESGGGLVQPGGSLRLSCAASGFTFSSYYMSWVRQAPGKGLEWVADISVSGSYTNYADSVKGRFTISRDNSKNTLYLQMNSLRAEDTAVYYCARIGSYRSFFSTDDGDSLDYWGQGTLVTVSSASTKGPSVFPLAPSSKSTSGGTAALGCLVKDYFPEPVTVSWNSGALTSGVHTFPAVLQSSGLYSLSSVVTVPSSSLGTQTYICNVNHKPSNTKVDKRVEPKSCDKTHTCPPCPAPEFEGGPSVFLFPPKPKDTLMISRTPEVTCVVVDVEHEDPEVKFNWYVDGVEVHNAKTKPREEQYNSTYRVVSVLTVLHQDWLNGKEYKCKVSNKALPASIEKTISKAKGQPREPQVYTLPPCRKKLTKNQVSLTCLVKGFYPSDIAVEWESNGQPENNYKTTPPVLKSDGSFFLYSKLTVDKSRWQQGNVFSCSVMHEALHNHYTQKSLSLSPGKGGGGSGGGGSNPQIAAHVISEASSKTTSVLQWAEKGYYTMSNNLVTLENGKQLTVKRQGLYYIYAQVTFCSNREASSQAPFIASLCLKSPGRFERILLRAANTHSSAKPCGQQSIHLGGVFELQPGASVFVNVTDPSQVSHGTGFTSFGLLKLGGGGSGGGGSNPQIAAHVISEASSKTTSVLQWAEKGYYTMSNNLVTLENGKQLTVKRQGLYYIYAQVTFCSNREASSQAPFIASLCLKSPGRFERILLRAANTHSSAKPCGQQSIHLGGVFELQPGASVFVNVTDPSQVSHGTGFTSFGLLKLGGGGSGGGGSNPQIAAHVISEASSKTTSVLQWAEKGYYTMSNNLVTLENGKQLTVKRQGLYYIYAQVTFCSNREASSQAPFIASLCLKSPGRFERILLRAANTHSSAKPCGQQSIHLGGVFELQPGASVFVNVTDPSQVSHGTGFTSFGLLKL

SEQ ID NO: 70 - protein, 725 aa, synthetic construct
  source 1..725: note = chain 1
EVQLLESGGGLVQPGGSLRLSCAASGFTFSSYYMSWVRQAPGKGLEWVADISVSGSYTNYADSVKGRFTISRDNSKNTLYLQMNSLRAEDTAVYYCARIGSYRSFFSTDDGDSLDYWGQGTLVTVSSASTKGPSVFPLAPSSKSTSGGTAALGCLVKDYFPEPVTVSWNSGALTSGVHTFPAVLQSSGLYSLSSVVTVPSSSLGTQTYICNVNHKPSNTKVDKRVEPKSCDKTHTCPPCPAPEFEGGPSVFLFPPKPKDTLMISRTPEVTCVVVDVEHEDPEVKFNWYVDGVEVHNAKTKPREEQYNSTYRVVSVLTVLHQDWLNGKEYKCKVSNKALPASIEKTISKAKGQPREPQVYTLPPSRDELTKNQVSLTCLVKGFYPSDIAVEWESNGQPENNYKTTPPVLDSDGSFFLYSKLTVDKSRWQQGNVFSCSVMHEALHNHYTQKSLSLSPGKGGGGSGGGGSGGGGSQVQLVQSGAEVKKPGASVKVSCKASGYTFTGYYMHWVRQAPGQGLEWMGWINPDSGGTNYAQKFQGRVTMTRDTSISTAYMELNRLRSDDTAVYYCARDQPLGYCTNGVCSYFDYWGQGTLVTVSSGGGGSGGGGSGGGGSGGGGSDIQMTQSPSSVSASVGDRVTITCRASQGIYSWLAWYQQKPGKAPNLLIYTASTLQSGVPSRFSGSGSGTDFTLTISSLQPEDFATYYCQQANIFPLTFGGGTKVEIK

SEQ ID NO: 71 - protein, 725 aa, synthetic construct
  source 1..725: note = chain 1
QVQLVQSGAEVKKPGASVKVSCKASGYTFTGYYMHWVRQAPGQGLEWMGWINPDSGGTNYAQKFQGRVTMTRDTSISTAYMELNRLRSDDTAVYYCARDQPLGYCTNGVCSYFDYWGQGTLVTVSSASTKGPSVFPLAPSSKSTSGGTAALGCLVKDYFPEPVTVSWNSGALTSGVHTFPAVLQSSGLYSLSSVVTVPSSSLGTQTYICNVNHKPSNTKVDKRVEPKSCDKTHTCPPCPAPEFEGGPSVFLFPPKPKDTLMISRTPEVTCVVVDVEHEDPEVKFNWYVDGVEVHNAKTKPREEQYNSTYRVVSVLTVLHQDWLNGKEYKCKVSNKALPASIEKTISKAKGQPREPQVYTLPPSRDELTKNQVSLTCLVKGFYPSDIAVEWESNGQPENNYKTTPPVLDSDGSFFLYSKLTVDKSRWQQGNVFSCSVMHEALHNHYTQKSLSLSPGKGGGGSGGGGSGGGGSEVQLLESGGGLVQPGGSLRLSCAASGFTFSSYYMSWVRQAPGKGLEWVADISVSGSYTNYADSVKGRFTISRDNSKNTLYLQMNSLRAEDTAVYYCARIGSYRSFFSTDDGDSLDYWGQGTLVTVSSGGGGSGGGGSGGGGSGGGGSDIQMTQSPSTLSASVGDRVTITCRASQSISSWLAWYQQKPGKAPKLLIYDASSLESGVPSRFSGSGSGTEFTLTISSLQPDDFATYYCQQYNSYSLTFGGGTKVEIK

SEQ ID NO: 72 - protein, 713 aa, synthetic construct
  source 1..713: note = chain 1
EVQLVESGGGLVQPGGSLRLSCAASGYSFTGYYIHWVRQAPGKGLEWVARVIPNAGGTSYNQKFKGRFTLSVDNSKNTAYLQMNSLRAEDTAVYYCAREGIYWWGQGTLVTVSSASTKGPSVFPLAPSSKSTSGGTAALGCLVKDYFPEPVTVSWNSGALTSGVHTFPAVLQSSGLYSLSSVVTVPSSSLGTQTYICNVNHKPSNTKVDKRVEPKSCDKTHTCPPCPAPEFEGGPSVFLFPPKPKDTLMISRTPEVTCVVVDVEHEDPEVKFNWYVDGVEVHNAKTKPREEQYNSTYRVVSVLTVLHQDWLNGKEYKCKVSNKALPASIEKTISKAKGQPREPQVYTLPPSRDELTKNQVSLTCLVKGFYPSDIAVEWESNGQPENNYKTTPPVLDSDGSFFLYSKLTVDKSRWQQGNVFSCSVMHEALHNHYTQKSLSLSPGKGGGGSGGGGSGGGGSEVQLLESGGGLVQPGGSLRLSCAASGFTFSSYYMSWVRQAPGKCLEWVADISVSGSYTNYADSVKGRFTISRDNSKNTLYLQMNSLRAEDTAVYYCARIGSYRSFFSTDDGDSLDYWGQGTLVTVSSGGGGSGGGGSGGGGSGGGGSDIQMTQSPSTLSASVGDRVTITCRASQSISSWLAWYQQKPGKAPKLLIYDASSLESGVPSRFSGSGSGTEFTLTISSLQPDDFATYYCQQYNSYSLTFGCGTKVEIK

SEQ ID NO: 73 - protein, 713 aa, synthetic construct
  source 1..713: note = chain 1
EVQLVESGGGLVQPGGSLRLSCAASGYSFTGYYIHWVRQAPGKGLEWVARVIPNAGGTSYNQKFKGRFTLSVDNSKNTAYLQMNSLRAEDTAVYYCAREGIYWWGQGTLVTVSSASTKGPSVFPLAPSSKSTSGGTAALGCLVKDYFPEPVTVSWNSGALTSGVHTFPAVLQSSGLYSLSSVVTVPSSSLGTQTYICNVNHKPSNTKVDKRVEPKSCDKTHTCPPCPAPEFEGGPSVFLFPPKPKDTLMISRTPEVTCVVVDVSHEDPEVKFNWYVDGVEVHNAKTKPREEQYNSTYRVVSVLTVLHQDWLNGKEYKCKVSNKALPASIEKTISKAKGQPREPQVYTLPPSRDELTKNQVSLTCLVKGFYPSDIAVEWESNGQPENNYKTTPPVLDSDGSFFLYSKLTVDKSRWQQGNVFSCSVMHEALHNHYTQKSLSLSPGKGGGGSGGGGSGGGGSEVQLLESGGGLVQPGGSLRLSCAASGFTFSSYYMSWVRQAPGKCLEWVADISVSGSYTNYADSVKGRFTISRDNSKNTLYLQMNSLRAEDTAVYYCARIGSYRSFFSTDDGDSLDYWGQGTLVTVSSGGGGSGGGGSGGGGSGGGGSDIQMTQSPSTLSASVGDRVTITCRASQSISSWLAWYQQKPGKAPKLLIYDASSLESGVPSRFSGSGSGTEFTLTISSLQPDDFATYYCQQYNSYSLTFGCGTKVEIK

SEQ ID NO: 74 - protein, 651 aa, synthetic construct
  source 1..651: note = chain 1
EVQLLESGGGLVQPGGSLRLSCAASGFTFSSYYMSWVRQAPGKGLEWVADISVSGSYTNYADSVKGRFTISRDNSKNTLYLQMNSLRAEDTAVYYCARIGSYRSFFSTDDGDSLDYWGQGTLVTVSSASTKGPSVFPLAPSSKSTSGGTAALGCLVKDYFPEPVTVSWNSGALTSGVHTFPAVLQSSGLYSLSSVVTVPSSSLGTQTYICNVNHKPSNTKVDKRVEPKSCDKTHTCPPCPAPEFEGGPSVFLFPPKPKDTLMISRTPEVTCVVVDVEHEDPEVKFNWYVDGVEVHNAKTKPREEQYNSTYRVVSVLTVLHQDWLNGKEYKCKVSNKALPASIEKTISKAKGQPREPQVYTLPPSRDELTKNQVSLTCLVKGFYPSDIAVEWESNGQPENNYKTTPPVLDSDGSFFLYSKLTVDKSRWQQGNVFSCSVMHEALHNHYTQKSLSLSPGKGGGGSGGGGSREGPELSPDDPAGLLDLRQGMFAQLVAQNVLLIDGPLSWYSDPGLAGVSLTGGLSYKEDTKELVVAKAGVYYVFFQLELRRVVAGEGSGSVSLALHLQPLRSAAGAAALALTVDLPPASSEARNSAFGFQGRLLHLSAGQRLGVHLHTEARARHAWQLTQGATVLGLFRVTPEIPAGLPSPRSE

SEQ ID NO: 75 - protein, 1039 aa, synthetic construct
  source 1..1039: note = chain 1
EVQLLESGGGLVQPGGSLRLSCAASGFTFSSYYMSWVRQAPGKGLEWVADISVSGSYTNYADSVKGRFTISRDNSKNTLYLQMNSLRAEDTAVYYCARIGSYRSFFSTDDGDSLDYWGQGTLVTVSSASTKGPSVFPLAPSSKSTSGGTAALGCLVKDYFPEPVTVSWNSGALTSGVHTFPAVLQSSGLYSLSSVVTVPSSSLGTQTYICNVNHKPSNTKVDKRVEPKSCDKTHTCPPCPAPEFEGGPSVFLFPPKPKDTLMISRTPEVTCVVVDVEHEDPEVKFNWYVDGVEVHNAKTKPREEQYNSTYRVVSVLTVLHQDWLNGKEYKCKVSNKALPASIEKTISKAKGQPREPQVYTLPPCRKKLTKNQVSLTCLVKGFYPSDIAVEWESNGQPENNYKTTPPVLKSDGSFFLYSKLTVDKSRWQQGNVFSCSVMHEALHNHYTQKSLSLSPGKGGGGSGGGGSREGPELSPDDPAGLLDLRQGMFAQLVAQNVLLIDGPLSWYSDPGLAGVSLTGGLSYKEDTKELVVAKAGVYYVFFQLELRRVVAGEGSGSVSLALHLQPLRSAAGAAALALTVDLPPASSEARNSAFGFQGRLLHLSAGQRLGVHLHTEARARHAWQLTQGATVLGLFRVTPEIPAGLPSPRSEGGGGSGGGGSREGPELSPDDPAGLLDLRQGMFAQLVAQNVLLIDGPLSWYSDPGLAGVSLTGGLSYKEDTKELVVAKAGVYYVFFQLELRRVVAGEGSGSVSLALHLQPLRSAAGAAALALTVDLPPASSEARNSAFGFQGRLLHLSAGQRLGVHLHTEARARHAWQLTQGATVLGLFRVTPEIPAGLPSPRSEGGGGSGGGGSREGPELSPDDPAGLLDLRQGMFAQLVAQNVLLIDGPLSWYSDPGLAGVSLTGGLSYKEDTKELVVAKAGVYYVFFQLELRRVVAGEGSGSVSLALHLQPLRSAAGAAALALTVDLPPASSEARNSAFGFQGRLLHLSAGQRLGVHLHTEARARHAWQLTQGATVLGLFRVTPEIPAGLPSPRSE

SEQ ID NO: 76 - protein, 722 aa, synthetic construct
  source 1..722: note = chain 1
EVQLLESGGGLVQPGGSLRLSCAASGFTFSSYYMSWVRQAPGKGLEWVADISVSGSYTNYADSVKGRFTISRDNSKNTLYLQMNSLRAEDTAVYYCARIGSYRSFFSTDDGDSLDYWGQGTLVTVSSASTKGPSVFPLAPSSKSTSGGTAALGCLVKDYFPEPVTVSWNSGALTSGVHTFPAVLQSSGLYSLSSVVTVPSSSLGTQTYICNVNHKPSNTKVDKRVEPKSCDKTHTCPPCPAPEFEGGPSVFLFPPKPKDTLMISRTPEVTCVVVDVSHEDPEVKFNWYVDGVEVHNAKTKPREEQYNSTYRVVSVLTVLHQDWLNGKEYKCKVSNKALPASIEKTISKAKGQPREPQVYTLPPSRDELTKNQVSLTCLVKGFYPSDIAVEWESNGQPENNYKTTPPVLDSDGSFFLYSKLTVDKSRWQQGNVFSCSVMHEALHNHYTQKSLSLSPGKGGGGSGGGGSGGGGSQVQLQQWGAGLLKPSETLSLTCAVYGGSFSGYYWSWIRQSPEKGLEWIGEINHGGYVTYNPSLESRVTISVDTSKNQFSLKLSSVTAADTAVYYCARDYGPGNYDWYFDLWGRGTLVTVSSGGGGSGGGGSGGGGSGGGGSEIVLTQSPATLSLSPGERATLSCRASQSVSSYLAWYQQKPGQAPRLLIYDASNRATGIPARFSGSGSGTDFTLTISSLEPEDFAVYYCQQRSNWPPALTFGGGTKVEIK

SEQ ID NO: 77 - protein, 716 aa, synthetic construct
  source 1..716: note = chain 1
EVQLLESGGGLVQPGGSLRLSCAASGFTFSSYYMSWVRQAPGKGLEWVADISVSGSYTNYADSVKGRFTISRDNSKNTLYLQMNSLRAEDTAVYYCARIGSYRSFFSTDDGDSLDYWGQGTLVTVSSASTKGPSVFPLAPSSKSTSGGTAALGCLVKDYFPEPVTVSWNSGALTSGVHTFPAVLQSSGLYSLSSVVTVPSSSLGTQTYICNVNHKPSNTKVDKRVEPKSCDKTHTCPPCPAPEFEGGPSVFLFPPKPKDTLMISRTPEVTCVVVDVEHEDPEVKFNWYVDGVEVHNAKTKPREEQYNSTYRVVSVLTVLHQDWLNGKEYKCKVSNKALPASIEKTISKAKGQPREPQVYTLPPSRDELTKNQVSLTCLVKGFYPSDIAVEWESNGQPENNYKTTPPVLDSDGSFFLYSKLTVDKSRWQQGNVFSCSVMHEALHNHYTQKSLSLSPGKGGGGSGGGGSGGGGSEVQLVQSGAEVKKPGESLRISCKGSGYSFSTYWISWVRQMPGKGLEWMGKIYPGDSYTNYSPSFQGQVTISADKSISTAYLQWSSLKASDTAMYYCARGYGIFDYWGQGTLVTVSSGGGGSGGGGSGGGGSGGGGSSYELTQPPSVSVSPGQTASITCSGDNIGDQYAHWYQQKPGQSPVLVIYQDKNRPSGIPERFSGSNSGNTATLTISGTQAMDEADYYCATYTGFGSLAVFGGGTKLTVL

SEQ ID NO: 78 - protein, 720 aa, synthetic construct
  source 1..720: note = chain 1
QVQLQQWGAGLLKPSETLSLTCAVYGGSFSGYYWSWIRQSPEKGLEWIGEINHGGYVTYNPSLESRVTISVDTSKNQFSLKLSSVTAADTAVYYCARDYGPGNYDWYFDLWGRGTLVTVSSASTKGPSVFPLAPSSKSTSGGTAALGCLVKDYFPEPVTVSWNSGALTSGVHTFPAVLQSSGLYSLSSVVTVPSSSLGTQTYICNVNHKPSNTKVDKRVEPKSCDKTHTCPPCPAPEFEGGPSVFLFPPKPKDTLMISRTPEVTCVVVDVSHEDPEVKFNWYVDGVEVHNAKTKPREEQYNSTYRVVSVLTVLHQDWLNGKEYKCKVSNKALPASIEKTISKAKGQPREPQVYTLPPSRDELTKNQVSLTCLVKGFYPSDIAVEWESNGQPENNYKTTPPVLDSDGSFFLYSKLTVDKSRWQQGNVFSCSVMHEALHNHYTQKSLSLSPGKGGGGSGGGGSGGGGSEVQLLESGGGLVQPGGSLRLSCAASGFTFSSYYMSWVRQAPGKGLEWVADISVSGSYTNYADSVKGRFTISRDNSKNTLYLQMNSLRAEDTAVYYCARIGSYRSFFSTDDGDSLDYWGQGTLVTVSSGGGGSGGGGSGGGGSGGGGSDIQMTQSPSTLSASVGDRVTITCRASQSISSWLAWYQQKPGKAPKLLIYDASSLESGVPSRFSGSGSGTEFTLTISSLQPDDFATYYCQQYNSYSLTFGGGTKVEIK

SEQ ID NO: 79 - protein, 715 aa, synthetic construct
  source 1..715: note = chain 1
EVQLVQSGAEVKKPGESLRISCKGSGYSFSTYWISWVRQMPGKGLEWMGKIYPGDSYTNYSPSFQGQVTISADKSISTAYLQWSSLKASDTAMYYCARGYGIFDYWGQGTLVTVSSASTKGPSVFPLAPSSKSTSGGTAALGCLVKDYFPEPVTVSWNSGALTSGVHTFPAVLQSSGLYSLSSVVTVPSSSLGTQTYICNVNHKPSNTKVDKRVEPKSCDKTHTCPPCPAPEFEGGPSVFLFPPKPKDTLMISRTPEVTCVVVDVEHEDPEVKFNWYVDGVEVHNAKTKPREEQYNSTYRVVSVLTVLHQDWLNGKEYKCKVSNKALPASIEKTISKAKGQPREPQVYTLPPSRDELTKNQVSLTCLVKGFYPSDIAVEWESNGQPENNYKTTPPVLDSDGSFFLYSKLTVDKSRWQQGNVFSCSVMHEALHNHYTQKSLSLSPGKGGGGSGGGGSGGGGSEVQLLESGGGLVQPGGSLRLSCAASGFTFSSYYMSWVRQAPGKGLEWVADISVSGSYTNYADSVKGRFTISRDNSKNTLYLQMNSLRAEDTAVYYCARIGSYRSFFSTDDGDSLDYWGQGTLVTVSSGGGGSGGGGSGGGGSGGGGSDIQMTQSPSTLSASVGDRVTITCRASQSISSWLAWYQQKPGKAPKLLIYDASSLESGVPSRFSGSGSGTEFTLTISSLQPDDFATYYCQQYNSYSLTFGGGTKVEIK

SEQ ID NO: 80 - protein, 457 aa, synthetic construct
  source 1..457: note = chain 2
EVQLLESGGGLVQPGGSLRLSCAASGFTFSSYYMSWVRQAPGKGLEWVADISVSGSYTNYADSVKGRFTISRDNSKNTLYLQMNSLRAEDTAVYYCARIGSYRSFFSTDDGDSLDYWGQGTLVTVSSASTKGPSVFPLAPSSKSTSGGTAALGCLVKDYFPEPVTVSWNSGALTSGVHTFPAVLQSSGLYSLSSVVTVPSSSLGTQTYICNVNHKPSNTKVDKRVEPKSCDKTHTCPPCPAPEFEGGPSVFLFPPKPKDTLMISRTPEVTCVVVDVSHEDPEVKFNWYVDGVEVHNAKTKPREEQYNSTYRVVSVLTVLHQDWLNGKEYKCKVSNKALPASIEKTISKAKGQPREPQVCTLPPSRDELTKNQVSLTCLVEGFYPSDIAVEWESNGQPENNYKTTPPVLDSDGSFFLYSDLTVDKSRWQQGNVFSCSVMHEALHNHYTQESLSLSPGK

SEQ ID NO: 81 - protein, 457 aa, synthetic construct
  source 1..457: note = chain 2
QVQLVESGGGLVKPGGSLRLSCAASGFTFSDYYMSWIRQAPGKGLEWVSDISVSSSYTNYADSVKGRFTISRDNAKNSLYLQMNSLRAEDTAVYYCARLGGYRSFFSTDDGDSLDYWGQGTLVTVSSASTKGPSVFPLAPSSKSTSGGTAALGCLVKDYFPEPVTVSWNSGALTSGVHTFPAVLQSSGLYSLSSVVTVPSSSLGTQTYICNVNHKPSNTKVDKRVEPKSCDKTHTCPPCPAPEFEGGPSVFLFPPKPKDTLMISRTPEVTCVVVDVSHEDPEVKFNWYVDGVEVHNAKTKPREEQYNSTYRVVSVLTVLHQDWLNGKEYKCKVSNKALPASIEKTISKAKGQPREPQVCTLPPSRDELTKNQVSLTCLVEGFYPSDIAVEWESNGQPENNYKTTPPVLDSDGSFFLYSDLTVDKSRWQQGNVFSCSVMHEALHNHYTQESLSLSPGK

SEQ ID NO: 82 - protein, 457 aa, synthetic construct
  source 1..457: note = chain 2
EVQLLESGGGLVQPGGSLRLSCAASGFTFSSYYMSWVRQAPGKGLEWVADISVSGSYTNYADSVKGRFTISRDNSKNTLYLQMNSLRAEDTAVYYCARIGSYRSFFSTDDGDSLDYWGQGTLVTVSSASTKGPSVFPLAPSSKSTSGGTAALGCLVKDYFPEPVTVSWNSGALTSGVHTFPAVLQSSGLYSLSSVVTVPSSSLGTQTYICNVNHKPSNTKVDKRVEPKSCDKTHTCPPCPAPEFEGGPSVFLFPPKPKDTLMISRTPEVTCVVVDVEHEDPEVKFNWYVDGVEVHNAKTKPREEQYNSTYRVVSVLTVLHQDWLNGKEYKCKVSNKALPASIEKTISKAKGQPREPQVCTLPPSRDELTKNQVSLTCLVEGFYPSDIAVEWESNGQPENNYKTTPPVLDSDGSFFLYSDLTVDKSRWQQGNVFSCSVMHEALHNHYTQESLSLSPGK

SEQ ID NO: 83 - protein, 214 aa, synthetic construct
  source 1..214: note = chain 3
DIQMTQSPSTLSASVGDRVTITCRASQSISSWLAWYQQKPGKAPKLLIYDASSLESGVPSRFSGSGSGTEFTLTISSLQPDDFATYYCQQYNSYSLTFGGGTKVEIKRTVAAPSVFIFPPSDEQLKSGTASVVCLLNNFYPREAKVQWKVDNALQSGNSQESVTEQDSKDSTYSLSSTLTLSKADYEKHKVYACEVTHQGLSSPVTKSFNRGEC

SEQ ID NO: 84 - protein, 214 aa, synthetic construct
  source 1..214: note = chain 3
DIQLTQSPSTLSASVGDRVTITCRASQSISSWLAWYQQKPGKAPKLLIYDAFSLESGVPSRFSGSGSGTEFTLTISSLQPDDFATYYCQQYNSYSITFGGGTKVEIKRTVAAPSVFIFPPSDEQLKSGTASVVCLLNNFYPREAKVQWKVDNALQSGNSQESVTEQDSKDSTYSLSSTLTLSKADYEKHKVYACEVTHQGLSSPVTKSFNRGEC

SEQ ID NO: 85 - protein, 214 aa, synthetic construct
  source 1..214: note = chain 3
DIQMTQSPSSVSASVGDRVTITCRASQGIYSWLAWYQQKPGKAPNLLIYTASTLQSGVPSRFSGSGSGTDFTLTISSLQPEDFATYYCQQANIFPLTFGGGTKVEIKRTVAAPSVFIFPPSDEQLKSGTASVVCLLNNFYPREAKVQWKVDNALQSGNSQESVTEQDSKDSTYSLSSTLTLSKADYEKHKVYACEVTHQGLSSPVTKSFNRGEC

SEQ ID NO: 86 - protein, 219 aa, synthetic construct
  source 1..219: note = chain 3
DIQMTQSPSSLSASVGDRVTITCRSSQSLVHSNGNTFLHWYQQKPGKAPKLLIYTVSNRFSGVPSRFSGSGSGTDFTLTISSLQPEDFATYFCSQTTHVPWTFGQGTKVEIKRTVAAPSVFIFPPSDEQLKSGTASVVCLLNNFYPREAKVQWKVDNALQSGNSQESVTEQDSKDSTYSLSSTLTLSKADYEKHKVYACEVTHQGLSSPVTKSFNRGEC

SEQ ID NO: 87 - protein, 216 aa, synthetic construct
  source 1..216: note = chain 3
EIVLTQSPATLSLSPGERATLSCRASQSVSSYLAWYQQKPGQAPRLLIYDASNRATGIPARFSGSGSGTDFTLTISSLEPEDFAVYYCQQRSNWPPALTFGGGTKVEIKRTVAAPSVFIFPPSDEQLKSGTASVVCLLNNFYPREAKVQWKVDNALQSGNSQESVTEQDSKDSTYSLSSTLTLSKADYEKHKVYACEVTHQGLSSPVTKSFNRGEC

SEQ ID NO: 88 - protein, 214 aa, synthetic construct
  source 1..214: note = chain 3
SYELTQPPSVSVSPGQTASITCSGDNIGDQYAHWYQQKPGQSPVLVIYQDKNRPSGIPERFSGSNSGNTATLTISGTQAMDEADYYCATYTGFGSLAVFGGGTKLTVLGQPKAAPSVTLFPPSSEELQANKATLVCLISDFYPGAVTVAWKADSSPVKAGVETTTPSKQSNNKYAASSYLSLTPEQWKSHRSYSCQVTHEGSTVEKTVAPTECS